European Patent Specification EP 3 760 208 B1, published May 29, 2024. Title: TARGETING HUMAN SATELLITE II (HSATII). Applicant: The General Hospital Corporation. Application PCT/US2015/037792. The sequence listing filed with the application follows.

SEQUENCE LISTING (29 sequences)

SEQ ID NO: 1 - DNA, 170 bp, Homo sapiens
ccattcgattccattcgatgattccattcgattccattcgatgatgattccattcgattccattcgatgattccattcgattccattcgatgatgattccattcgattccattcgatgattccattcgattccattcgatgatgattccattcgattccattcgatgatt

SEQ ID NO: 2 - DNA, 23 bp, Artificial Sequence
  oligo target sequence
ccattcgattccattcgatgatt

SEQ ID NO: 3 - DNA, 26 bp, Artificial Sequence
  oligo target sequence
ccattcgattccattcgatgatgatt

SEQ ID NO: 4 - DNA, 49 bp, Artificial Sequence
  oligo target sequence
ccattcgattccattcgatgattccattcgattccattcgatgatgatt

SEQ ID NO: 5 - DNA, 21 bp, Artificial Sequence
  oligo target sequence
cattcgattccattcgatgat

SEQ ID NO: 6 - DNA, 21 bp, Artificial Sequence
  oligo target sequence
atcatcgaatggaatcgaatg

SEQ ID NO: 7 - DNA, 21 bp, Artificial Sequence
  synthetically generated oligonucleotide
cattcgattccattcgatgat

SEQ ID NO: 8 - DNA, 21 bp, Artificial Sequence
  synthetically generated oligonucleotide
atcatcgaatggaatcgaatg

SEQ ID NO: 9 - DNA, 21 bp, Artificial Sequence
  synthetically generated oligonucleotide
cgcgcttctcgttggggtctt

SEQ ID NO: 10 - DNA, 21 bp, Artificial Sequence
  synthetically generated oligonucleotide
aagaccccaacgagaagcgcg

SEQ ID NO: 11 - DNA, 22 bp, Artificial Sequence
  synthetically generated oligonucleotide
ttgcgtgtcatccttgcgcagg

SEQ ID NO: 12 - DNA, 23 bp, Artificial Sequence
  synthetically generated oligonucleotide
gcattcaattcattagatgacgg

SEQ ID NO: 13 - DNA, 20 bp, Artificial Sequence
  synthetically generated oligonucleotide
ccttgacccgaatgcaatca

SEQ ID NO: 14 - DNA, 24 bp, Artificial Sequence
  synthetically generated oligonucleotide
tctaaccctaactgagaagggcgt

SEQ ID NO: 15 - DNA, 24 bp, Artificial Sequence
  synthetically generated oligonucleotide
tgctctagaatgaacggtggaagg

SEQ ID NO: 16 - DNA, 20 bp, Artificial Sequence
  synthetically generated oligonucleotide
ccattcgttaatgcctttcg

SEQ ID NO: 17 - DNA, 20 bp, Artificial Sequence
  synthetically generated oligonucleotide
cacgaatggaatcattgtcg

SEQ ID NO: 18 - DNA, 20 bp, Artificial Sequence
  synthetically generated oligonucleotide
tccattcgaggattccactc

SEQ ID NO: 19 - DNA, 21 bp, Artificial Sequence
  synthetically generated oligonucleotide
caaagggaagcaaaggaaatc

SEQ ID NO: 20 - DNA, 20 bp, Artificial Sequence
  synthetically generated oligonucleotide
ggggtaaaagggcatgtttt

SEQ ID NO: 21 - DNA, 20 bp, Artificial Sequence
  synthetically generated oligonucleotide
ctgaagaagcccactcaagg

SEQ ID NO: 22 - DNA, 20 bp, Artificial Sequence
  synthetically generated oligonucleotide
ctcttccagccttccttcct

SEQ ID NO: 23 - DNA, 20 bp, Artificial Sequence
  synthetically generated oligonucleotide
agcactgtgttggcgtacag

SEQ ID NO: 24 - DNA, 16 bp, Artificial Sequence
  synthetically generated oligonucleotide
gattccattcgatgat

SEQ ID NO: 25 - DNA, 17 bp, Artificial Sequence
  synthetically generated oligonucleotide
atggaatcatcatcgaa

SEQ ID NO: 26 - DNA, 17 bp, Artificial Sequence
  synthetically generated oligonucleotide
tggaatcatcgaatgga

SEQ ID NO: 27 - DNA, 15 bp, Artificial Sequence
  synthetically generated oligonucleotide
aacacgtctatacgc

SEQ ID NO: 28 - DNA, 21 bp, Artificial Sequence
  synthetically generated oligonucleotide
gtccagatgaagctcccagaa

SEQ ID NO: 29 - DNA, 21 bp, Artificial Sequence
  synthetically generated oligonucleotide
caccatccactacaactacat